European Patent Specification EP 3 990 646 B1, published March 5, 2025. Title: Mammalian cell lines with SIRT-1 gene knockout. Applicant: F. Hoffmann-La Roche AG Hoffmann-La Roche Inc. The sequence listing filed with the application follows.

SEQUENCE LISTING (18 sequences)

SEQ ID NO: 1 - DNA, 34 bp, Artificial Sequence
  L3
ataacttcgtataaagtctcctatacgaagttat

SEQ ID NO: 2 - DNA, 34 bp, Artificial Sequence
  2L
ataacttcgtatagcatacattatacgaagttat

SEQ ID NO: 3 - DNA, 34 bp, Artificial Sequence
  loxFas
acaacttcgtatatacctttctatacgaagttgt

SEQ ID NO: 4 - DNA, 608 bp, Human cytomegalovirus
gttgacattgattattgactagttattaatagtaatcaattacggggtcattagttcatagcccatatatggagttccgcgttacataacttacggtaaatggcccgcctggctgaccgcccaacgacccccgcccattgacgtcaataatgacgtatgttcccatagtaacgccaatagggactttccattgacgtcaatgggtggagtatttacggtaaactgcccacttggcagtacatcaagtgtatcatatgccaagtacgccccctattgacgtcaatgacggtaaatggcccgcctggcattatgcccagtacatgaccttatgggactttcctacttggcagtacatctacgtattagtcatcgctattagcatggtgatgcggttttggcagtacatcaatgggcgtggatagcggtttgactcacggggatttccaagtctccaccccattgacgtcaatgggagtttgttttggcaccaaaatcaacgggactttccaaaatgtcgtaacaactccgccccattgacgcaaatgggcggtaggcgtgtacggtgggaggtctatataagcagagctccgtttagtgaacgtcagatc

SEQ ID NO: 5 - DNA, 696 bp, Human cytomegalovirus
gttgacattgattattgactagttattaatagtaatcaattacggggtcattagttcatagcccatatatggagttccgcgttacataacttacggtaaatggcccgcctggctgaccgcccaacgacccccgcccattgacgtcaataatgacgtatgttcccatagtaacgccaatagggactttccattgacgtcaatgggtggagtatttacggtaaactgcccacttggcagtacatcaagtgtatcatatgccaagtacgccccctattgacgtcaatgacggtaaatggcccgcctggcattatgcccagtacatgaccttatgggactttcctacttggcagtacatctacgtattagtcatcgctattagcatggtgatgcggttttggcagtacatcaatgggcgtggatagcggtttgactcacggggatttccaagtctccaccccattgacgtcaatgggagtttgttttggcaccaaaatcaacgggactttccaaaatgtcgtaacaactccgccccattgacgcaaatgggcggtaggcgtgtacggtgggaggtctatataagcagagctccgtttagtgaacgtcagatctagctctgggagaggagcccagcactagaagtcggcggtgtttccattcggtgatcagcactgaacacagaggaagcttgccgccacc

SEQ ID NO: 6 - DNA, 2125 bp, Human cytomegalovirus
ctgcagtgaataataaaatgtgtgtttgtccgaaatacgcgttttgagatttctgtcgccgactaaattcatgtcgcgcgatagtggtgtttatcgccgatagagatggcgatattggaaaaatcgatatttgaaaatatggcatattgaaaatgtcgccgatgtgagtttctgtgtaactgatatcgccatttttccaaaagtgatttttgggcatacgcgatatctggcgatagcgcttatatcgtttacgggggatggcgatagacgactttggtgacttgggcgattctgtgtgtcgcaaatatcgcagtttcgatataggtgacagacgatatgaggctatatcgccgatagaggcgacatcaagctggcacatggccaatgcatatcgatctatacattgaatcaatattggccattagccatattattcattggttatatagcataaatcaatattggctattggccattgcatacgttgtatccatatcataatatgtacatttatattggctcatgtccaacattaccgccatgttgacattgattattgactagttattaatagtaatcaattacggggtcattagttcatagcccatatatggagttccgcgttacataacttacggtaaatggcccgcctggctgaccgcccaacgacccccgcccattgacgtcaataatgacgtatgttcccatagtaacgccaatagggactttccattgacgtcaatgggtggagtatttacggtaaactgcccacttggcagtacatcaagtgtatcatatgccaagtacgccccctattgacgtcaatgacggtaaatggcccgcctggcattatgcccagtacatgaccttatgggactttcctacttggcagtacatctacgtattagtcatcgctattaccatggtgatgcggttttggcagtacatcaatgggcgtggatagcggtttgactcacggggatttccaagtctccaccccattgacgtcaatgggagtttgttttggcaccaaaatcaacgggactttccaaaatgtcgtaacaactccgccccattgacgcaaatgggcggtaggcgtgtacggtgggaggtctatataagcagagctcgtttagtgaaccgtcagatcgcctggagacgccatccacgctgttttgacctccatagaagacaccgggaccgatccagcctccgcggccgggaacggtgcattggaacgcggattccccgtgccaagagtgacgtaagtaccgcctatagagtctataggcccacccccttggcttcttatgcatgctatactgtttttggcttggggtctatacacccccgcttcctcatgttataggtgatggtatagcttagcctataggtgtgggttattgaccattattgaccactcccctattggtgacgatactttccattactaatccataacatggctctttgccacaactctctttattggctatatgccaatacactgtccttcagagactgacacggactctgtatttttacaggatggggtctcatttattatttacaaattcacatatacaacaccaccgtccccagtgcccgcagtttttattaaacataacgtgggatctccacgcgaatctcgggtacgtgttccggacatgggctcttctccggtagcggcggagcttctacatccgagccctgctcccatgcctccagcgactcatggtcgctcggcagctccttgctcctaacagtggaggccagacttaggcacagcacgatgcccaccaccaccagtgtgccgcacaaggccgtggcggtagggtatgtgtctgaaaatgagctcggggagcgggcttgcaccgctgacgcatttggaagacttaaggcagcggcagaagaagatgcaggcagctgagttgttgtgttctgataagagtcagaggtaactcccgttgcggtgctgttaacggtggagggcagtgtagtctgagcagtactcgttgctgccgcgcgcgccaccagacataatagctgacagactaacagactgttcctttccatgggtcttttctgcagtcaccgtccttgacacggtttaaacgccgccacc

SEQ ID NO: 7 - DNA, 129 bp, Simian virus 40
aacttgtttattgcagcttataatggttacaaataaagcaatagcatcacaaatttcacaaataaagcatttttttcaccattctagttgtggtttgtccaaactcatcaatgtatcttatcatgtctg

SEQ ID NO: 8 - DNA, 225 bp, Bos taurus
ctgtgccttctagttgccagccatctgttgtttgcccctcccccgtgccttccttgaccctggaaggtgccactcccactgtcctttcctaataaaatgaggaaattgcatcgcattgtctgagtaggtgtcattctattctggggggtggggtggggcaggacagcaagggggaggattgggaagacaatagcaggcatgctggggatgcggtgggctctatgg

SEQ ID NO: 9 - DNA, 73 bp, Homo sapiens
caggataatatatggtagggttcatagccagagtaacctttttttttaatttttattttattttatttttgag

SEQ ID NO: 10 - DNA, 288 bp, Simian virus 40
agtcagcaaccaggtgtggaaagtccccaggctccccagcaggcagaagtatgcaaagcatgcatctcaattagtcagcaaccatagtcccgcccctaactccgcccatcccgcccctaactccgcccagttccgcccattctccgccccatggctgactaattttttttatttatgcagaggccgaggccgcctctgcctctgagctattccagaagtagtgaggaggcttttttggaggcctaggcttttgcaaaaagctcccgggagcttgtatatccattttcg

SEQ ID NO: 11 - DNA, 798 bp, Artificial Sequence
  green fluorescent protein encoding nucleic acid
atggtgagcaagggcgaggagctgttcaccggggtggtgcccatcctggtcgagctggacggcgacgtaaacggccacaagttcagcgtgtccggcgagggcgagggcgatgccacctacggcaagctgaccctgaagttcatctgcaccaccggcaagctgcccgtgccctggcccaccctcgtgaccaccctgacctacggcgtgcagtgcttcagccgctaccccgaccacatgaagcagcacgacttcttcaagtccgccatgcccgaaggctacgtccaggagcgcaccatcttcttcaaggacgacggcaactacaagacccgcgccgaggtgaagttcgagggcgacaccctggtgaaccgcatcgagctgaagggcatcgacttcaaggaggacggcaacatcctggggcacaagctggagtacaactacaacagccacaacgtctatatcatggccgacaagcagaagaacggcatcaaggtgaacttcaagatccgccacaacatcgaggacggcagcgtgcagctcgccgaccactaccagcagaacacccccatcggcgacggccccgtgctgctgcccgacaaccactacctgagcacccagtccgccctgagcaaagaccccaacgagaagcgcgatcacatggtcctgctggagttcgtgaccgccgccgggatcactctcggcatggacgagctgtacaagtccggactcagatctcgagctcaagcttcgaattctgcagtcgacggtaccgcgggcccgggatccaccggatctagatga

SEQ ID NO: 12 - DNA, 20 bp, Artificial Sequence
  gRNA_SIRT1_1
tatcatccaactcaggtgga

SEQ ID NO: 13 - DNA, 20 bp, Artificial Sequence
  gRNA_SIRT1_2
gcagcatctcatgattggca

SEQ ID NO: 14 - DNA, 20 bp, Artificial Sequence
  gRNA_SIRT1_3
gcattcttgaagtaacttca

SEQ ID NO: 15 - DNA, 20 bp, Artificial Sequence
  oSA060_SIRT1_for
gctgcccttcaagttatggc

SEQ ID NO: 16 - DNA, 20 bp, Artificial Sequence
  oSA061_SIRT1_rev
gctggccttttgactcacag

SEQ ID NO: 17 - protein, 747 aa, Homo sapiens
MADEAALALQPGGSPSAAGADREAASSPAGEPLRKRPRRDGPGLERSPGEPGGAAPEREVPAAARGCPGAAAAALWREAEAEAAAAGGEQEAQATAAAGEGDNGPGLQGPSREPPLADNLYDEDDDDEGEEEEEAAAAAIGYRDNLLFGDEIITNGFHSCESDEEDRASHASSSDWTPRPRIGPYTFVQQHLMIGTDPRTILKDLLPETIPPPELDDMTLWQIVINILSEPPKRKKRKDINTIEDAVKLLQECKKIIVLTGAGVSVSCGIPDFRSRDGIYARLAVDFPDLPDPQAMFDIEYFRKDPRPFFKFAKEIYPGQFQPSLCHKFIALSDKEGKLLRNYTQNIDTLEQVAGIQRIIQCHGSFATASCLICKYKVDCEAVRGDIFNQVVPRCPRCPADEPLAIMKPEIVFFGENLPEQFHRAMKYDKDEVDLLIVIGSSLKVRPVALIPSSIPHEVPQILINREPLPHLHFDVELLGDCDVIINELCHRLGGEYAKLCCNPVKLSEITEKPPRTQKELAYLSELPPTPLHVSEDSSSPERTSPPDSSVIVTLLDQAAKSNDDLDVSESKGCMEEKPQEVQTSRNVESIAEQMENPDLKNVGSSTGEKNERTSVAGTVRKCWPNRVAKEQISRRLDGNQYLFLPPNRYIFHGAEVYSDSEDDVLSSSSCGSNSDSGTCQSPSLEEPMEDESEIEEFYNGLEDEPDVPERAGGAGFGTDGDDQEAINEAISVKQEVTDMNYPSNKS

SEQ ID NO: 18 - protein, 693 aa, Cricetulus griseus
MEAASQPADEPLRKSAQRRAWPRAQPGRVEPGGRGGGGGAAAAAAGCEAASAAAPAAALWREAVGAAAAGAEQEARRPPRPGRKQWVGPAAGAEGCRRLRRRRGRGGRRGGGGGGGGSDRLPRFSFSGIGPYTFVQQHLMIGTDPRTILKDLLPETIPPPELDDMTLWQIVINILSEPPKRKKRKDINTIEDAVKLLQECKKIIVLTGAGVSVSCGIPDFRSRDGIYARLAVDFPDLPDPQAMFDIEYFRKDPRPFFKFAKEIYPGQFQPSLCHKFIALSDKEGKLLRNYTQNIDTLEQVAGIQRIIQCHGSFATASCLICKYKVDCETVRGDIFNQVVPRCPRCPADEPLAIMKPEIVFFGENLPEQFHRAMKYDKDEVDLLIVIGSSLKVRPVALIPSSIPHEVPQILINREPLPHLHFDVELLGDCDVIINELCHRLGGEYAKLCCNPVKLSEITEKPPRTQKELVHLSELPPTPLHISEDSSSPERTVPQDSASMIATCVDQATENRVDLEVSESEGCVEEKSQEAQTCRSVESINVENPDLKAVGSSTGEKNERTSVAEAVRKCWPNRLAKEQISKRLDGNQYLFVPPNRYIFHGAEVYSDSEDDILSSSSCGSNSDSGTCQSPSLEEPMEDESEIEEFYNGLEDDTDRPEGTGGSGLGVDGGEQELVHEATAMRQEATDVNYPSDKS